European Patent Specification EP 3 893 934 B1, published September 10, 2025. Title: Insulin conjugate. Applicant: Sanofi. The sequence listing filed with the application follows.

SEQUENCE LISTING (105 sequences)

SEQ ID NO: 1 - protein, 21 aa, Homo sapiens
  Chain A
GIVEQCCTSICSLYQLENYCN

SEQ ID NO: 2 - protein, 30 aa, Homo sapiens
  Chain B
FVNQHLCGSHLVEALYLVCGERGFFYTPKT

SEQ ID NO: 3 - protein, 21 aa, Artificial Sequence
  Chain A
GIVEQCCTSICSLEQLENYCN

SEQ ID NO: 4 - protein, 29 aa, Artificial Sequence
  Chain B
FVNQHLCGSHLVEALYLVCGERGFFYTPK

SEQ ID NO: 5 - protein, 21 aa, Artificial Sequence
  Chain A
GIVEQCCTSICSLYQLENYCN

SEQ ID NO: 6 - protein, 29 aa, Artificial Sequence
  Chain B
FVNQHLCGSHLVEALLLVCGERGFFYTPK

SEQ ID NO: 7 - protein, 21 aa, Artificial Sequence
  Chain A
GIVEQCCTSICSLYQLENYCG

SEQ ID NO: 8 - protein, 29 aa, Artificial Sequence
  Chain B
FVNQHLCGSHLVEALWLVCGERGFFYTPK

SEQ ID NO: 9 - protein, 21 aa, Artificial Sequence
  Chain A
GIVEQCCTSICSLYQLENYCN

SEQ ID NO: 10 - protein, 29 aa, Artificial Sequence
  Chain B
FVNQHLCGSHLVEALHLVCGERGFFYTPK

SEQ ID NO: 11 - protein, 21 aa, Artificial Sequence
  Chain A
GIVEQCCTSICSLYQLENYCN

SEQ ID NO: 12 - protein, 29 aa, Artificial Sequence
  Chain B
FVNQHLCGSHLVEALVLVCGERGFFYTPK

SEQ ID NO: 13 - protein, 21 aa, Artificial Sequence
  Chain A
GIVEQCCTSICSLYQLENYCN

SEQ ID NO: 14 - protein, 30 aa, Artificial Sequence
  Chain B
FVNQHLCGSHLVEALYLVCGERGFAYTPKT

SEQ ID NO: 15 - protein, 21 aa, Artificial Sequence
  Chain A
GIVEQCCTSICSLYQLENYCN

SEQ ID NO: 16 - protein, 29 aa, Artificial Sequence
  Chain B
FVNQHLCGSHLVEALYLVCGERGFAYTPK

SEQ ID NO: 17 - protein, 21 aa, Artificial Sequence
  Chain A
GIVEQCCTSICSLYQLENYCN

SEQ ID NO: 18 - protein, 29 aa, Artificial Sequence
  Chain B
FVNQHLCGSHLVEALYLVCGERGFEYTPK

SEQ ID NO: 19 - protein, 21 aa, Artificial Sequence
  Chain A
GIVEQCCTSICSLYQLENYCN

SEQ ID NO: 20 - protein, 29 aa, Artificial Sequence
  Chain B
FVNQHLCGSHLVEALYLVCGERGFHYTPK

SEQ ID NO: 21 - protein, 21 aa, Artificial Sequence
  Chain A
GIVEQCCTSICSLYQLENYCN

SEQ ID NO: 22 - protein, 29 aa, Artificial Sequence
  Chain B
FVNQHLCGSHLVEALYLVCGERGFLYTPK

SEQ ID NO: 23 - protein, 21 aa, Artificial Sequence
  Chain A
GIVEQCCTSICSLYQLENYCN

SEQ ID NO: 24 - protein, 29 aa, Artificial Sequence
  Chain B
FVNQHLCGSHLVEALYLVCGERGFVYTPK

SEQ ID NO: 25 - protein, 21 aa, Artificial Sequence
  Chain A
GIVEQCCTSICSLYQLENYCN

SEQ ID NO: 26 - protein, 29 aa, Artificial Sequence
  Chain B
FVNQHLCGSHLVEALHLVCGERGFHYTPK

SEQ ID NO: 27 - protein, 21 aa, Artificial Sequence
  Chain A
GIVEQCCTSICSLYQLENYCG

SEQ ID NO: 28 - protein, 29 aa, Artificial Sequence
  Chain B
FVNQHLCGSHLVEALWLVCGERGFHYTPK

SEQ ID NO: 29 - protein, 21 aa, Artificial Sequence
  Chain A
GIVEQCCTSICSLYQLENYCG

SEQ ID NO: 30 - protein, 29 aa, Artificial Sequence
  Chain B
FVNQHLCGSHLVEALWLVCGERGFWYTPK

SEQ ID NO: 31 - protein, 21 aa, Artificial Sequence
  Chain A
GIVEQCCTSICSLEQLENYCN

SEQ ID NO: 32 - protein, 29 aa, Artificial Sequence
  Chain B
FVNQHLCGSHLVEALHLVCGERGFFYTPK

SEQ ID NO: 33 - protein, 21 aa, Artificial Sequence
  Chain A
GIVEQCCTSICSLEQLENYCG

SEQ ID NO: 34 - protein, 29 aa, Artificial Sequence
  Chain B
FVNQHLCGSHLVEALWLVCGERGFFYTPK

SEQ ID NO: 35 - protein, 21 aa, Artificial Sequence
  Chain A
GIVEQCCTSICSLEQLENYCN

SEQ ID NO: 36 - protein, 29 aa, Artificial Sequence
  Chain B
FVNQHLCGSHLVEALILVCGERGFFYTPK

SEQ ID NO: 37 - protein, 21 aa, Artificial Sequence
  Chain A
GIVEQCCTSICSLEQLENYCN

SEQ ID NO: 38 - protein, 29 aa, Artificial Sequence
  Chain B
FVNQHLCGSHLVEALVLVCGERGFFYTPK

SEQ ID NO: 39 - protein, 21 aa, Artificial Sequence
  Chain A
GIVEQCCTSICSLEQLENYCN

SEQ ID NO: 40 - protein, 29 aa, Artificial Sequence
  Chain B
FVEQHLCGSHLVEALVLVCGERGFFYTPK

SEQ ID NO: 41 - protein, 21 aa, Artificial Sequence
  Chain A
GIVEQCCTSICSLEQLENYCN

SEQ ID NO: 42 - protein, 29 aa, Artificial Sequence
  Chain B
FVNQHLCGSHLVEALYLVCGERGFHYTPK

SEQ ID NO: 43 - protein, 21 aa, Artificial Sequence
  Chain A
GIVEQCCTSICSLEQLENYCN

SEQ ID NO: 44 - protein, 29 aa, Artificial Sequence
  Chain B
FVNQHLCGSHLVEALYLVCGERGFIYTPK

SEQ ID NO: 45 - protein, 21 aa, Artificial Sequence
  Chain A
GIVEQCCTSICSLEQLENYCG

SEQ ID NO: 46 - protein, 29 aa, Artificial Sequence
  Chain B
FVNQHLCGSHLVEALYLVCGERGFWYTPK

SEQ ID NO: 47 - protein, 21 aa, Artificial Sequence
  Chain A
GIVEQCCTSICSLEQLENYCN

SEQ ID NO: 48 - protein, 29 aa, Artificial Sequence
  Chain B
FVNQHLCGSHLVEALYLVCGERGFVYTPK

SEQ ID NO: 49 - protein, 21 aa, Artificial Sequence
  Chain A
GIVEQCCTSICSLEQLENYCG

SEQ ID NO: 50 - protein, 29 aa, Artificial Sequence
  Chain B
FVEQHLCGSHLVEALYLVCGERGFVYTPK

SEQ ID NO: 51 - protein, 21 aa, Artificial Sequence
  Chain A
GIVEQCCTSICSLEQLENYCN

SEQ ID NO: 52 - protein, 29 aa, Artificial Sequence
  Chain B
FVNQHLCGSHLVEALELVCGERGFHYTPK

SEQ ID NO: 53 - protein, 21 aa, Artificial Sequence
  Chain A
GIVEQCCTSICSLEQLENYCN

SEQ ID NO: 54 - protein, 29 aa, Artificial Sequence
  Chain B
FVNQHLCGSHLVEALHLVCGERGFAYTPK

SEQ ID NO: 55 - protein, 21 aa, Artificial Sequence
  Chain A
GIVEQCCTSICSLEQLENYCN

SEQ ID NO: 56 - protein, 29 aa, Artificial Sequence
  Chain B
FVNQHLCGSHLVEALHLVCGERGFHYTPK

SEQ ID NO: 57 - protein, 21 aa, Artificial Sequence
  Chain A
GIVEQCCTSICSLEQLENYCN

SEQ ID NO: 58 - protein, 29 aa, Artificial Sequence
  Chain B
FVNQHLCGSHLVEALILVCGERGFIYTPK

SEQ ID NO: 59 - protein, 21 aa, Artificial Sequence
  Chain A
GIVEQCCTSICSLEQLENYCN

SEQ ID NO: 60 - protein, 29 aa, Artificial Sequence
  Chain B
FVEQHLCGSHLVEALILVCGERGFIYTPK

SEQ ID NO: 61 - protein, 21 aa, Artificial Sequence
  Chain A
GIVEQCCTSICSLEQLENYCG

SEQ ID NO: 62 - protein, 29 aa, Artificial Sequence
  Chain B
FVEQHLCGSHLVEALILVCGERGFWYTPK

SEQ ID NO: 63 - protein, 21 aa, Artificial Sequence
  Chain A
GIVEQCCTSICSLEQLENYCN

SEQ ID NO: 64 - protein, 29 aa, Artificial Sequence
  Chain B
FVNQHLCGSHLVEALILVCGERGFVYTPK

SEQ ID NO: 65 - protein, 21 aa, Artificial Sequence
  Chain A
GIVEQCCTSICSLEQLENYCG

SEQ ID NO: 66 - protein, 29 aa, Artificial Sequence
  Chain B
FVEQHLCGSHLVEALILVCGERGFVYTPK

SEQ ID NO: 67 - protein, 21 aa, Artificial Sequence
  Chain A
GIVEQCCTSICSLEQLENYCN

SEQ ID NO: 68 - protein, 29 aa, Artificial Sequence
  Chain B
FVNQHLCGSHLVEALLLVCGERGFAYTPK

SEQ ID NO: 69 - protein, 21 aa, Artificial Sequence
  Chain A
GIVEQCCTSICSLEQLENYCN

SEQ ID NO: 70 - protein, 29 aa, Artificial Sequence
  Chain B
FVNQHLCGSHLVEALVLVCGERGFIYTPK

SEQ ID NO: 71 - protein, 21 aa, Artificial Sequence
  Chain A
GIVEQCCTSICSLEQLENYCG

SEQ ID NO: 72 - protein, 29 aa, Artificial Sequence
  Chain B
FVNQHLCGSHLVEALVLVCGERGFWYTPK

SEQ ID NO: 73 - protein, 21 aa, Artificial Sequence
  Chain A
GIVEQCCTSICSLEQLENYCG

SEQ ID NO: 74 - protein, 29 aa, Artificial Sequence
  Chain B
FVEQHLCGSHLVEALVLVCGERGFWYTPK

SEQ ID NO: 75 - protein, 21 aa, Artificial Sequence
  Chain A
GIVEQCCTSICSLEQLENYCN

SEQ ID NO: 76 - protein, 29 aa, Artificial Sequence
  Chain B
FVNQHLCGSHLVEALVLVCGERGFVYTPK

SEQ ID NO: 77 - protein, 21 aa, Artificial Sequence
  Chain A
GIVEQCCTSICSLEQLENYCN

SEQ ID NO: 78 - protein, 29 aa, Artificial Sequence
  Chain B
FVEQHLCGSHLVEALVLVCGERGFVYTPK

SEQ ID NO: 79 - protein, 21 aa, Artificial Sequence
  Chain A
GIVEQCCTSICSLEQLENYCG

SEQ ID NO: 80 - protein, 29 aa, Artificial Sequence
  Chain B
FVEQHLCGSHLVEALVLVCGERGFVYTPK

SEQ ID NO: 81 - protein, 21 aa, Bos
  Chain A
GIVEQCCASVCSLYQLENYCN

SEQ ID NO: 82 - protein, 30 aa, Bos
  Chain B
FVNQHLCGSHLVEALYLVCGERGFFYTPKA

SEQ ID NO: 83 - protein, 21 aa, Sus
  Chain A
GIVEQCCTSICSLYQLENYCN

SEQ ID NO: 84 - protein, 30 aa, Sus; identical to SEQ ID NO: 82
  Chain B

SEQ ID NO: 85 - protein, 29 aa, Artificial Sequence
  Chain B
FVNQHLCGSHLVEALYLVCGERGFLYTPK

SEQ ID NO: 86 - protein, 29 aa, Artificial Sequence
  Chain B
FVNQHLCGSHLVEALYLVCGERGFVYTPK

SEQ ID NO: 87 - protein, 29 aa, Artificial Sequence
  Chain B
FVNQHLCGSHLVEALYLVCGERGFIYTPK

SEQ ID NO: 88 - protein, 29 aa, Artificial Sequence
  Chain B
FVNQHLCGSHLVEALYLVCGERGFVYTPK

SEQ ID NO: 89 - protein, 29 aa, Artificial Sequence
  Chain B
FVEQHLCGSHLVEALYLVCGERGFVYTPK

SEQ ID NO: 90 - protein, 29 aa, Artificial Sequence
  Chain B
FVNQHLCGSHLVEALILVCGERGFIYTPK

SEQ ID NO: 91 - protein, 29 aa, Artificial Sequence
  Chain B
FVEQHLCGSHLVEALILVCGERGFIYTPK

SEQ ID NO: 92 - protein, 29 aa, Artificial Sequence
  Chain B
FVNQHLCGSHLVEALILVCGERGFVYTPK

SEQ ID NO: 93 - protein, 29 aa, Artificial Sequence
  Chain B
FVEQHLCGSHLVEALILVCGERGFVYTPK

SEQ ID NO: 94 - protein, 29 aa, Artificial Sequence
  Chain B
FVNQHLCGSHLVEALVLVCGERGFIYTPK

SEQ ID NO: 95 - protein, 29 aa, Artificial Sequence
  Chain B
FVNQHLCGSHLVEALVLVCGERGFVYTPK

SEQ ID NO: 96 - protein, 29 aa, Artificial Sequence
  Chain B
FVEQHLCGSHLVEALVLVCGERGFVYTPK

SEQ ID NO: 97 - protein, 29 aa, Artificial Sequence
  Chain B
FVEQHLCGSHLVEALVLVCGERGFVYTPK

SEQ ID NO: 98 - protein, 44 aa, Artificial Sequence
  Lixisenatide
HGEGTFTSDLSKQMEEEAVRLFIEWLKNGGPSSGAPPSKKKKKK

SEQ ID NO: 99 - protein, 39 aa, Artificial Sequence
  Exenatide
HGEGTFTSDLSKQMEEEAVRLFIEWLKNGGPSSGAPPPS

SEQ ID NO: 100 - protein, 31 aa, Artificial Sequence
  Semaglutide
  MOD_RES 2: Aib
HAEGTFTSDVSSYLEGQAAKEFIAWLVRGRG

SEQ ID NO: 101 - protein, 31 aa, Artificial Sequence
  Dulaglutide
HAEGTFTSDVSSYLEGQAAKEFIAWLVKGRG

SEQ ID NO: 102 - protein, 21 aa, Homo sapiens
  human insulin , A chain
GIVEQCCTSICSLYQLENYCN

SEQ ID NO: 103 - protein, 30 aa, Homo sapiens; identical to SEQ ID NO: 2
  human insulin , B chain

SEQ ID NO: 104 - protein, 21 aa, Artificial Sequence
  insulin analog 1 , A chain
GIVEQCCTSICSLEQLENYCN

SEQ ID NO: 105 - protein, 29 aa, Artificial Sequence
  insulin analog 1 , B chain
FVNQHLCGSHLVEALHLVCGERGFHYTPK